European Patent Application EP 4 317 446 A1, published February 7, 2024. Title: Recombinant chimeric adenovirus vector substituted with the knob gene of chimpanzee adenovirus serotype 6 and use of the same. Applicant: GENEMATRIX INC. The sequence listing filed with the application follows.

SEQUENCE LISTING (62 sequences)

SEQ ID NO: 1 - protein, 173 aa, Artificial Sequence
  Chimpanzee adenovirus serotype 6 Fiber knob domain a.a sequence(synthesized ChAdV-6 knob a.a sequences are underlined)
PDPSPNCQLLSDRDAKFTLCLTKCGSQILGTVAVAAVTVGSALNPINDTVKSAIVFLRFDSDGVLMSNSSMVGDYWNFREGQTTQSVAYTNAVGFMPNIGAYPKTQSKTPKNSIVSQVYLTGETTMPMTLTITFNGTDEKDTTPVSTYSMTFTWQWTGDYKDKNITFATNSFS

SEQ ID NO: 2 - DNA, 519 bp, Artificial Sequence
  Chimpanzee adenovirus serotype 6/Pan6/Sad23 Fiber knob domain nucleotide sequence
cctgacccaagccctaattgtcaattactttcagacagagatgccaaatttactctctgtcttacaaaatgcggtagtcaaatactaggcactgtggcagtggcggctgttactgtaggatcagcactaaatccaattaatgacacagtcaaaagcgccatagttttccttagatttgattccgatggtgtactcatgtcaaactcatcaatggtaggtgattactggaactttagggagggacagaccactcaaagtgtagcctatacaaatgctgtgggattcatgccaaatataggtgcatatccaaaaacccaaagtaaaacacctaaaaatagcatagtcagtcaggtatatttaactggagaaactactatgccaatgacactaaccataactttcaatggcactgatgaaaaagacacaaccccagttagcacctactctatgacttttacatggcagtggactggagactataaggacaaaaatattacctttgctaccaactcattctct

SEQ ID NO: 3 - protein, 318 aa, Artificial Sequence
  Chimeric hexon HVR 1 to 7 region a.a sequence (HAdV-5 hexon + HAdV-28 HVR 1-7 region)
SSQWDAQEKSGQGSDMVTKTHTFGQAPYSGINITKEGIQIGTEITADNQKKEIFADKTFQPEPQIGEENWQENEVFYGGRVLKKTTPMKPCYGSYAKPTNENGGQAKFKTPAEGQEPKELDIDLAFFDTDGGTADTEYKADIVLYSEDVDIETPDTHISYMPGKEDDSSEINLVQQSMPNRPNYIAFRDNFIGLMYYNSTGNMGVLAGQASQLNAVVDLQDRNTELSYQLLLDSIGDRTRYFSMWNQAVDSYDPDVRIIENHGTEDELPNYCFPLDGLGTNATYQGVKVSTGDGATQSGWAKDDTMARQNQICRGNIY

SEQ ID NO: 4 - DNA, 954 bp, Artificial Sequence
  Chimeric hexon HVR 1 to 7 region nucleotide sequence (HAdV-5 hexon + HAdV-28 HVR 1-7 region)
tccagtcagtgggatgcgcaagaaaaaagtggacaaggaagtgacatggttactaaaactcacacatttgggcaggcgccttattctggtataaatattacaaaggagggtattcaaataggtactgaaattaccgccgacaatcaaaagaaagaaatttttgccgataaaacatttcaacctgaacctcaaataggagaagagaactggcaagaaaatgaagtcttctatggcgggagagtcctaaaaaagactaccccaatgaaaccatgttacggttcatatgcaaaacccacaaatgaaaatggagggcaagcaaaattcaaaacacctgctgaaggacaggaacctaaagaacttgacattgaccttgcttttttcgacactgacggcggaacagctgacactgaatataaagcagatattgtattgtacagtgaagatgtagatatagaaaccccagacactcatatttcttacatgcccggcaaggaagatgacagttcagaaatcaatctagttcaacaatctatgcccaacaggcctaattacattgcttttagggacaattttattggtctaatgtattacaacagcacgggtaatatgggtgttctggcgggccaagcatcgcagttgaatgctgttgtagatttgcaagacagaaacacagagctttcataccagcttttgcttgattccattggtgatagaaccaggtacttttctatgtggaatcaggctgttgacagctatgatccagatgttagaattattgaaaatcatggaactgaagatgaacttccaaattactgctttccactggacggattgggaactaatgctacctatcaaggtgtaaaagtatcaactggagatggtgctacgcaaagcggatgggcaaaagacgacacaatggccaggcaaaaccaaatatgcaggggtaacatctac

SEQ ID NO: 5 - DNA, 1731 bp, Artificial Sequence
  Chimeric fiber gene sequence (HAdV-5 tail, shift domain + ChAdV-6 knob domain)
atgaagcgcgcaagaccgtctgaagataccttcaaccccgtgtatccatatgacacggaaaccggtcctccaactgtgccttttcttactcctccctttgtatcccccaatgggtttcaagagagtccccctggggtactctctttgcgcctatccgaacctctagttacctccaatggcatgcttgcgctcaaaatgggcaacggcctctctctggacgaggccggcaaccttacctcccaaaatgtaaccactgtgagcccacctctcaaaaaaaccaagtcaaacataaacctggaaatatctgcacccctcacagttacctcagaagccctaactgtggctgccgccgcacctctaatggtcgcgggcaacacactcaccatgcaatcacaggccccgctaaccgtgcacgactccaaacttagcattgccacccaaggacccctcacagtgtcagaaggaaagctagccctgcaaacatcaggccccctcaccaccaccgatagcagtacccttactatcactgcctcaccccctctaactactgccactggtagcttgggcattgacttgaaagagcccatttatacacaaaatggaaaactaggactaaagtacggggctcctttgcatgtaacagacgacctaaacactttgaccgtagcaactggtccaggtgtgactattaataatacttccttgcaaactaaagttactggagccttgggttttgattcacaaggcaatatgcaacttaatgtagcaggaggactaaggattgattctcaaaacagacgccttatacttgatgttagttatccgtttgatgctcaaaaccaactaaatctaagactaggacagggccctctttttataaactcagcccacaacttggatattaactacaacaaaggcctttacttgtttacagcttcaaacaattccaaaaagcttgaggttaacctaagcactgccaaggggttgatgtttgacgctacagccatagccattaatgcaggagatgggcttgaatttggttcacctaatgcaccaaacacaaatcccctcaaaacaaaaattggccatggcctagaatttgattcaaacaaggctatggttcctaaactaggaactggccttagttttgacagcacaggtgccattacagtaggaaacaaaaataatgataagctaactttgtggaccacacctgacccaagccctaattgtcaattactttcagacagagatgccaaatttactctctgtcttacaaaatgcggtagtcaaatactaggcactgtggcagtggcggctgttactgtaggatcagcactaaatccaattaatgacacagtcaaaagcgccatagttttccttagatttgattccgatggtgtactcatgtcaaactcatcaatggtaggtgattactggaactttagggagggacagaccactcaaagtgtagcctatacaaatgctgtgggattcatgccaaatataggtgcatatccaaaaacccaaagtaaaacacctaaaaatagcatagtcagtcaggtatatttaactggagaaactactatgccaatgacactaaccataactttcaatggcactgatgaaaaagacacaaccccagttagcacctactctatgacttttacatggcagtggactggagactataaggacaaaaatattacctttgctaccaactcattctct

SEQ ID NO: 6 - DNA, 2832 bp, Artificial Sequence
  Chimeric hexon gene sequence (HAdV-5 hexon + HAdV-28 HVR 1-7region)
atggctaccccttcgatgatgccgcagtggtcttacatgcacatctcgggccaggacgcctcggagtacctgagccccgggctggtgcagtttgcccgcgccaccgagacgtacttcagcctgaataacaagtttagaaaccccacggtggcgcctacgcacgacgtgaccacagaccggtcccagcgtttgacgctgcggttcatccctgtggaccgtgaggatactgcgtactcgtacaaggcgcggttcaccctagctgtgggtgataaccgtgtgctggacatggcttccacgtactttgacatccgcggcgtgctggacaggggccctacttttaagccctactctggcactgcctacaacgccctggctcccaagggtgccccaaattccagtcagtgggatgcgcaagaaaaaagtggacaaggaagtgacatggttactaaaactcacacatttgggcaggcgccttattctggtataaatattacaaaggagggtattcaaataggtactgaaattaccgccgacaatcaaaagaaagaaatttttgccgataaaacatttcaacctgaacctcaaataggagaagagaactggcaagaaaatgaagtcttctatggcgggagagtcctaaaaaagactaccccaatgaaaccatgttacggttcatatgcaaaacccacaaatgaaaatggagggcaagcaaaattcaaaacacctgctgaaggacaggaacctaaagaacttgacattgaccttgcttttttcgacactgacggcggaacagctgacactgaatataaagcagatattgtattgtacagtgaagatgtagatatagaaaccccagacactcatatttcttacatgcccggcaaggaagatgacagttcagaaatcaatctagttcaacaatctatgcccaacaggcctaattacattgcttttagggacaattttattggtctaatgtattacaacagcacgggtaatatgggtgttctggcgggccaagcatcgcagttgaatgctgttgtagatttgcaagacagaaacacagagctttcataccagcttttgcttgattccattggtgatagaaccaggtacttttctatgtggaatcaggctgttgacagctatgatccagatgttagaattattgaaaatcatggaactgaagatgaacttccaaattactgctttccactggacggattgggaactaatgctacctatcaaggtgtaaaagtatcaactggagatggtgctacgcaaagcggatgggcaaaagacgacacaatggccaggcaaaaccaaatatgcaggggtaacatctacgccatggaaatcaatctaaatgccaacctgtggagaaatttcctgtactccaacatagcgctgtatttgcccgacaagctaaagtacagtccttccaacgtaaaaatttctgataacccaaacacctacgactacatgaacaagcgagtggtggctcccgggctagtggactgctacattaaccttggagcacgctggtcccttgactatatggacaacgtcaacccatttaaccaccaccgcaatgctggcctgcgctaccgctcaatgttgctgggcaatggtcgctatgtgcccttccacatccaggtgcctcagaagttctttgccattaaaaacctccttctcctgccgggctcatacacctacgagtggaacttcaggaaggatgttaacatggttctgcagagctccctaggaaatgacctaagggttgacggagccagcattaagtttgatagcatttgcctttacgccaccttcttccccatggcccacaacaccgcctccacgcttgaggccatgcttagaaacgacaccaacgaccagtcctttaacgactatctctccgccgccaacatgctctaccctatacccgccaacgctaccaacgtgcccatatccatcccctcccgcaactgggcggctttccgcggctgggccttcacgcgccttaagactaaggaaaccccatcactgggctcgggctacgacccttattacacctactctggctctataccctacctagatggaaccttttacctcaaccacacctttaagaaggtggccattacctttgactcttctgtcagctggcctggcaatgaccgcctgcttacccccaacgagtttgaaattaagcgctcagttgacggggagggttacaacgttgcccagtgtaacatgaccaaagactggttcctggtacaaatgctagctaactataacattggctaccagggcttctatatcccagagagctacaaggaccgcatgtactccttctttagaaacttccagcccatgagccgtcaggtggtggatgatactaaatacaaggactaccaacaggtgggcatcctacaccaacacaacaactctggatttgttggctaccttgcccccaccatgcgcgaaggacaggcctaccctgctaacttcccctatccgcttataggcaagaccgcagttgacagcattacccagaaaaagtttctttgcgatcgcaccctttggcgcatcccattctccagtaactttatgtccatgggcgcactcacagacctgggccaaaaccttctctacgccaactccgcccacgcgctagacatgacttttgaggtggatcccatggacgagcccacccttctttatgttttgtttgaagtctttgacgtggtccgtgtgcaccagccgcaccgcggcgtcatcgaaaccgtgtacctgcgcacgcccttctcggccggcaacgccacaacataa

SEQ ID NO: 7 - protein, 1270 aa, Artificial Sequence
  SARS-CoV-2_B.1.351(beta) spike modified amino acid sequence
MFVFLVLLPLVSSQCVNFTTRTQLPPAYTNSFTRGVYYPDKVFRSSVLHSTQDLFLPFFSNVTWFHAIHVSGTNGTKRFANPVLPFNDGVYFASTEKSNIIRGWIFGTTLDSKTQSLLIVNNATNVVIKVCEFQFCNDPFLGVYYHKNNKSWMESEFRVYSSANNCTFEYVSQPFLMDLEGKQGNFKNLREFVFKNIDGYFKIYSKHTPINLVRGLPQGFSALEPLVDLPIGINITRFQTLHISYLTPGDSSSGWTAGAAAYYVGYLQPRTFLLKYNENGTITDAVDCALDPLSETKCTLKSFTVEKGIYQTSNFRVQPTESIVRFPNITNLCPFGEVFNATRFASVYAWNRKRISNCVADYSVLYNSASFSTFKCYGVSPTKLNDLCFTNVYADSFVIRGDEVRQIAPGQTGNIADYNYKLPDDFTGCVIAWNSNNLDSKVGGNYNYLYRLFRKSNLKPFERDISTEIYQAGSTPCNGVKGFNCYFPLQSYGFQPTYGVGYQPYRVVVLSFELLHAPATVCGPKKSTNLVKNKCVNFNFNGLTGTGVLTESNKKFLPFQQFGRDIADTTDAVRDPQTLEILDITPCSFGGVSVITPGTNTSNQVAVLYQGVNCTEVPVAIHADQLTPTWRVYSTGSNVFQTRAGCLIGAEHVNNSYECDIPIGAGICASYQTQTNSPQQAQSVASQSIIAYTMSLGVENSVAYSNNSIAIPTNFTISVTTEILPVSMTKTSVDCTMYICGDSTECSNLLLQYGSFCTQLNRALTGIAVEQDKNTQEVFAQVKQIYKTPPIKDFGGFNFSQILPDPSKPSKRSFIEDLLFNKVTLADAGFIKQYGDCLGDIAARDLICAQKFNGLTVLPPLLTDEMIAQYTSALLAGTITSGWTFGAGAALQIPFAMQMAYRFNGIGVTQNVLYENQKLIANQFNSAIGKIQDSLSSTASALGKLQDVVNQNAQALNTLVKQLSSNFGAISSVLNDILSRLDPPEAEVQIDRLITGRLQSLQTYVTQQLIRAAEIRASANLAATKMSECVLGQSKRVDFCGKGYHLMSFPQSAPHGVVFLHVTYVPAQEKNFTTAPAICHDGKAHFPREGVFVSNGTHWFVTQRNFYEPQIITTDNTFVSGNCDVVIGIVNNTVYDPLQPELDSFKEELDKYFKNHTSPDVDLGDISGINASVVNIQKEIDRLNEVAKNLNESLIDLQELGKYEQYIKWPWYIWLGFIAGLIAIVMVTIMLCCMTSCCSCLKGCCSCGSCCKFDEDDSEPVLKGVKLHYT

SEQ ID NO: 8 - DNA, 3813 bp, Artificial Sequence
  SARS-CoV-2_B.1.351(beta) spike modified nucleic acid sequence
atgtttgtgtttctggtgctgctgcctctggtgagcagccagtgcgtgaacttcaccaccagaacccagctgcctcctgcctacaccaacagctttaccagaggcgtgtattaccccgacaaagtgtttagatcctccgtgctgcacagcacccaggacctgtttctgccctttttcagcaacgtgacctggttccatgccatccacgtgagcggcaccaacggcaccaagagattcgccaatcccgtgctgccttttaatgacggcgtgtactttgccagcaccgagaagagcaatatcatcagaggctggatcttcggcaccaccctggatagcaagacccagagcctgctgatcgtgaataatgccaccaatgtggtgatcaaagtgtgcgagttccagttttgtaacgacccctttctgggcgtgtattaccacaagaacaacaaaagctggatggagagcgaattcagagtgtacagcagcgccaataactgcacctttgagtacgtgagccagccctttctgatggacctggagggcaagcagggcaacttcaagaacctgagagagttcgtgtttaaaaatatcgacggctacttcaagatctacagcaagcatacacccatcaacctggtgagaggcctgccccagggcttcagcgccctggagcccctggtggacctgcccatcggcatcaacattacccggtttcagaccctgcacagaagctatctgacccccggcgacagcagcagcggctggaccgccggagccgccgcctattatgtgggctacctgcagcccagaaccttcctgctgaaatacaacgagaacggcaccatcaccgacgccgtggactgcgccctggaccccctgagcgagaccaagtgtaccctgaagagctttaccgtggagaagggcatctaccagaccagcaactttagagtgcagcccaccgagagcatcgtgagatttcccaacatcaccaacctgtgccccttcggggaggtgtttaatgccaccagattcgccagcgtgtacgcctggaatagaaaaagaatcagcaactgcgtggccgactacagcgtgctgtacaactctgccagcttttccacctttaagtgctacggcgtgagcccaaccaaactgaacgacctgtgcttcaccaacgtgtacgccgacagcttcgtgatcagaggcgacgaggtgagacagatcgcccccggccagaccggcaatatcgccgattacaactacaagctgcccgacgactttaccggctgcgtgatcgcctggaacagcaacaacctggacagcaaggtgggcggcaactacaactacctgtacagactgtttagaaagagcaacctgaagccctttgagagagacatcagcaccgagatctaccaggccggcagcaccccctgcaacggcgtgaaaggctttaattgttacttcccactgcagtcctacggcttccagcctacctacggcgtgggatatcagccctatagagtggtggtgctgtccttcgagctgctgcacgcccccgccaccgtgtgcggcccaaagaagagcaccaacctggtgaagaacaagtgcgtgaacttcaacttcaacggcctgaccggcaccggcgtgctgaccgagtccaacaagaaatttctgcccttccagcagttcggaagagacattgccgataccaccgacgccgtgagagacccccagaccctggagatcctggacatcaccccctgtagcttcggcggcgtgtccgtgatcaccccaggcaccaacacctccaaccaggtggccgtgctgtaccagggcgtgaactgtaccgaggtgcctgtggccatccacgccgatcagctgaccccaacctggagagtgtactccaccggctccaacgtgttccagaccagagccggctgtctgatcggcgccgagcacgtgaacaactcctacgagtgcgacatccctatcggcgccggcatctgcgccagctaccagacccagaccaatagcccccagcaggcccagtccgtggccagccagtccatcattgcctacaccatgtccctgggcgtggagaacagcgtggcctactccaacaacagcatcgccatccccaccaatttcaccatcagcgtgaccaccgaaatcctgccagtgagcatgaccaaaacctccgtggattgcaccatgtacatctgcggagactccaccgagtgctccaacctgctgctgcagtacggctccttttgcacccagctgaacagagccctgaccggaatcgccgtggagcaggataaaaacacccaggaagtgttcgcccaggtgaaacagatctacaagaccccccccatcaaagattttggaggctttaattttagccagatcctgcctgatccctccaaacccagcaagagatcctttatcgaggatctgctgttcaacaaagtgacactggccgatgccggatttatcaaacagtacggagactgcctgggcgacatcgccgccagagacctgatctgcgcccagaagtttaacggcctgaccgtgctgccacccctgctgaccgacgagatgatcgcccagtatacctccgccctgctggccggcaccatcacctccggctggacctttggcgccggagccgccctgcagatcccatttgccatgcagatggcctacagatttaatggaatcggagtgacccagaacgtgctgtatgagaaccagaaactgatcgccaatcagttcaacagcgccatcggcaagatccaggattctctgagctccaccgcctctgccctgggcaagctgcaggacgtggtgaatcagaacgcccaggccctgaacaccctggtgaaacagctgagcagcaactttggcgccatcagcagcgtgctgaatgatatcctgagcagactggatcctccagaggccgaggtgcagatcgacagactgatcacagggagactgcagagcctgcagacctatgtgacacagcagctgatcagagccgccgaaattagagccagcgccaacctggccgccaccaaaatgagcgagtgtgtgctgggacagagcaaaagagtggacttctgcggcaaaggctaccatctgatgagcttcccccagagcgccccccacggcgtggtgttcctgcatgtgacctacgtgcccgcccaggaaaaaaattttaccaccgcccctgccatctgtcacgacggcaaagcccattttcccagagagggcgtgtttgtgagcaacggcacccactggtttgtgacccagagaaacttttacgaaccccagatcatcaccacagataatacctttgtgagcggaaattgtgatgtggtgatcggcatcgtgaataataccgtgtatgatcctctgcagccagagctggacagctttaaggaggagctggacaagtattttaaaaatcataccagccccgacgtggatctgggagatatcagcggaatcaacgcctccgtggtgaatatccagaaggagatcgacagactgaacgaggtggccaaaaatctgaatgagtccctgatcgacctgcaggagctgggcaaatatgaacagtacatcaagtggccatggtacatctggctggggtttatcgccggactgatcgccatcgtgatggtgaccatcatgctgtgttgcatgaccagctgttgtagctgtctgaaaggctgttgtagctgcggcagctgctgcaaatttgacgaggatgattccgagccagtgctgaagggagtgaaactgcactatacctga

SEQ ID NO: 9 - protein, 138 aa, Artificial Sequence
  Sequence bound to the N-terminus of SARS-CoV-2-B.1.1.351 Spike protein
MGLPNNTASWFTALTQHGKEDLKFPRGQGVPINTNSSPDDQIGYYRRATRRIRGGDGKMKDLSPRWYFYYLGTGPEAGLPYGANKDGIIWVATEGALNTPKDHIGTRNPANNAAIVLQLPQGTTLPKGFYAEGSRGGS

SEQ ID NO: 10 - protein, 118 aa, Artificial Sequence [sequence omitted]

SEQ ID NO: 11 - DNA, 414 bp, Artificial Sequence
  Gene coding polypeptide bound to the N-terminus of SARS-CoV-2-B.1.1.351 Spike protein
atgggcctgcccaacaacaccgccagctggtttaccgccctgacccagcacggcaaggaggacctgaagttccccagaggccagggcgtgcccattaacaccaacagcagccccgacgaccagatcggctactacagaagagccaccagaagaatcagaggcggcgacggcaagatgaaggacctgagccccagatggtacttctactatctgggaaccggccccgaagccggcctgccctatggcgccaacaaagatggcatcatctgggtggccaccgaaggcgccctgaacacccccaaggatcacatcggaaccagaaatcccgccaacaatgccgccatcgtgctgcagctgccccagggaaccaccctgcctaaaggcttttatgccgaaggaagcagaggaggaagc

SEQ ID NO: 12 - DNA, 357 bp, Artificial Sequence
  Gene coding polypeptide bound to the C-terminus of SARS-CoV-2-B.1.1.351 Spike protein
accaaaaagagcgccgccgaggccagcaaaaagcccagacagaaaagaaccgccaccaaggcctacaatgtgacccaggcctttggcagaagaggacccgagcagacccagggcaattttggcgaccaggagctgatcagacagggcaccgactacaaacactggccccagatcgcccagttcgcccccagcgccagcgccttcttcggcatgagcagaatcggcatggaggtgacccccagcggcacctggctgacctacaccggcgccatcaagctggacgacaaggaccccaacttcaaggaccaggtgatcctgctgaacaagcacatcgacgcctacaagaccttcccctga

SEQ ID NO: 13 - protein, 494 aa, Artificial Sequence
  Human papillomavirus type 16, E6, E7 & Human papillomavirus type 18, E6, E7 modified amino acid sequence
MHQKRTAMFQDPQERPRKLPQLCTELQTTIHDIILECVYCKQQLLRREVYDFAFRDLCIVYRDGNPYAVCDKCLKFYSKISEYRHYCYSLYGTTLEQQYNKPLCDLLIRCIKQRHLDKKQRFHNIRGRWTGRCMSCCRSSRTRRETQLMHGDTPTLHEYMLDLQPETTQLNDSSEEEDEIDGPAGQAEPDRAHYNIVTFCCKCDSTLRLCVQSTHVDIRTLEDLLMGTLGIVCPICSQKPRGRKRRSMARFEDPTRRPYKLPDLCTELNTSLQDIEITCVYCKTVLELTEVFEFAFKDLFVVYRDSIPHAACHKCIDFYSRIRELRHYSDSVYGDTLEKLTNTGLYNLLIRCLKLRHLNEKRRFHNIAGHYRGQCHSCCNRARQERLQRRRETQVMHGPKATLQDIVLHLEPQNEIPVQLSDSEEENDEIDGVNHQHLPARRAEPQRHTMLCMCCKCEARIELVVESSADDLRAFQQLFLNTLSFVCPWCASQQ

SEQ ID NO: 14 - DNA, 1482 bp, Artificial Sequence
  Human papillomavirus type 16, E6, E7 & Human papillomavirus type 18, E6, E7 modified nucleic acid sequence
atgcaccagaagagaacagccatgttccaggaccctcaggaacggccacggaagctcccacaactttgtacagagctgcaaacaaccattcatgacatcatccttgaatgcgtttactgcaagcagcaacttctgcgccgggaagtctacgatttcgctttcagagatctgtgcatcgtgtatagagacgggaacccctacgccgtgtgtgacaaatgccttaaattctacagtaagatttcagagtaccggcattattgctacagcctttatggaactacattggagcagcagtacaacaaacctttgtgcgatcttcttatccggtgcattaagcaacggcacttggacaaaaaacaacggttccataacatcaggggcaggtggactggacgctgcatgagttgctgtcgctcaagccgcactcggagagagactcaactgatgcatggtgatactccaactttgcacgaatatatgttggacctccaacccgaaactacccaactgaatgacagctctgaggaagaggacgaaatcgacggccctgcagggcaagccgaacctgacagggcccattataacattgtgacattttgctgcaaatgcgatagtactttgagactctgtgtgcagtcaactcatgttgacattagaacacttgaagacctcctcatggggacactggggattgtttgcccaatctgttcacagaaacccagaggccgcaaaaggcggtctatggctcgctttgaggaccctacaaggaggccctacaagctccccgatttgtgtacagaactgaataccagtcttcaggatattgaaatcacttgcgtctactgcaaaactgtgctcgaacttaccgaagtctttgaatttgccttcaaggacctttttgttgtgtatcgcgattcaatcccacacgcagcctgtcacaaatgtattgacttctactctaggatcagagaattgaggcactattcagactctgtgtatggcgacaccttggaaaaattgaccaacactggattgtataatctgcttattcggtgtcttaagctccggcacttgaacgaaaaacgcagattccacaacattgccgggcattatcgcgggcaatgccattcttgttgcaatcgcgcccgccaggagcggctgcaaaggcgcagagagactcaggtgatgcatggacccaaggccactctccaggacatcgtccttcatcttgaaccccagaacgaaattcccgttcaacttagcgactcagaagaagaaaatgatgaaatcgacggagtgaaccatcagcatctcccagcaagaagagccgagccacaaagacacacaatgctctgtatgtgctgcaagtgtgaagcacggatcgaactcgtcgtcgaatctagtgcagatgatctcagagcctttcaacagctcttcttgaatacactgagctttgtctgtccatggtgcgctagtcaacaa

SEQ ID NO: 15 - protein, 37 aa, Artificial Sequence
  HVR1
PCEWDEAATALEINLEEEDDDNEDEVDEQAEQQKTHV

SEQ ID NO: 16 - protein, 8 aa, Artificial Sequence
  HVR2
VEGQTPKY

SEQ ID NO: 17 - protein, 12 aa, Artificial Sequence
  HVR3
SQWYETEINHAA

SEQ ID NO: 18 - protein, 18 aa, Artificial Sequence
  HVR4
GILVKQQNGKLESQVEMQ

SEQ ID NO: 19 - protein, 17 aa, Artificial Sequence
  HVR5
STTEATAGNGDNLTPKV

SEQ ID NO: 20 - protein, 12 aa, Artificial Sequence
  HVR6
TIKEGNSRELMG

SEQ ID NO: 21 - protein, 41 aa, Artificial Sequence
  HVR7
GGVINTETLTKVKPKTGQENGWEKDATEFSDKNEIRVGNNF

SEQ ID NO: 22 - protein, 22 aa, Artificial Sequence
  HVR1
SSQWDAQEKSGQGSDMVTKTHT

SEQ ID NO: 23 - protein, 13 aa, Artificial Sequence
  HVR2
TEITADNQKKEIF

SEQ ID NO: 24 - protein, 11 aa, Artificial Sequence
  HVR3
ENWQENEVFYG

SEQ ID NO: 25 - protein, 24 aa, Artificial Sequence
  Primer
GTAACCGCATACGAGCAGACGGTG

SEQ ID NO: 26 - protein, 15 aa, Artificial Sequence
  HVR5
DTDGGTADTEYKADI

SEQ ID NO: 27 - protein, 12 aa, Artificial Sequence
  HVR6
GKEDDSSEINLV

SEQ ID NO: 28 - protein, 43 aa, Artificial Sequence
  HVR7
DGLGTNATYQGVKVSTGDGATQSGWAKDDTMARQNQICRGNIY

SEQ ID NO: 29 - DNA, 33 bp, Artificial Sequence
  Primer
taagggtgggaaagaatatataaggtgggggtc

SEQ ID NO: 30 - DNA, 22 bp, Artificial Sequence
  Primer
gccttccatcaagggcatcccg

SEQ ID NO: 31 - DNA, 26 bp, Artificial Sequence
  Primer
gtaaagttccaagaagcgcgggatgc

SEQ ID NO: 32 - DNA, 25 bp, Artificial Sequence
  Primer
agttaatctcctggttcaccgtctg

SEQ ID NO: 33 - DNA, 24 bp, Artificial Sequence
  Primer
gtaaccgcatacgagcagacggtg

SEQ ID NO: 34 - DNA, 19 bp, Artificial Sequence
  Primer
cgtggagcggaaggtcacg

SEQ ID NO: 35 - DNA, 25 bp, Artificial Sequence
  Primer
gccagacatgatgcaagaccccgtg

SEQ ID NO: 36 - DNA, 31 bp, Artificial Sequence
  Primer
cgtaccactgagattctcctatttgaggttc

SEQ ID NO: 37 - DNA, 30 bp, Artificial Sequence
  Primer
caacctgaacctcaaataggagaatctcag

SEQ ID NO: 38 - DNA, 29 bp, Artificial Sequence
  Primer
ggataacgatctaaaggcgaacttcaaac

SEQ ID NO: 39 - DNA, 24 bp, Artificial Sequence
  Primer
gtcaggcagtagtttgaagttcgc

SEQ ID NO: 40 - DNA, 42 bp, Artificial Sequence
  Primer
ctctagttataactagaggatcttgatgtaatccagggttag

SEQ ID NO: 41 - DNA, 44 bp, Artificial Sequence
  Primer
cctctagttataactagagtacccgggatcttattccctttaac

SEQ ID NO: 42 - DNA, 28 bp, Artificial Sequence
  Primer
cggagtaacttgtatgtgttgggaattg

SEQ ID NO: 43 - DNA, 28 bp, Artificial Sequence
  Primer
caattcccaacacatacaagttactccg

SEQ ID NO: 44 - DNA, 40 bp, Artificial Sequence
  Primer
tatattctttcccacccttacgcgttaagatacattgatg

SEQ ID NO: 45 - DNA, 39 bp, Artificial Sequence
  Primer
cctttgctaccaactcattctctttttcatacattgccc

SEQ ID NO: 46 - DNA, 40 bp, Artificial Sequence
  Primer
acaattagggcttgggtcaggtgtggtccacaaagttagc

SEQ ID NO: 47 - DNA, 40 bp, Artificial Sequence
  Primer
gctaactttgtggaccacacctgacccaagccctaattgt

SEQ ID NO: 48 - DNA, 39 bp, Artificial Sequence
  Primer
gggcaatgtatgaaaaagagaatgagttggtagcaaagg

SEQ ID NO: 49 - DNA, 40 bp, Artificial Sequence
  Primer
tgcaggggtaacatctacgccatggaaatcaatctaaatg

SEQ ID NO: 50 - DNA, 40 bp, Artificial Sequence
  Primer
tgcgcatcccactgactggaatttggggcacccttgggag

SEQ ID NO: 51 - DNA, 40 bp, Artificial Sequence
  Primer
ctcccaagggtgccccaaattccagtcagtgggatgcgca

SEQ ID NO: 52 - DNA, 40 bp, Artificial Sequence
  Primer
catttagattgatttccatggcgtagatgttacccctgca

SEQ ID NO: 53 - DNA, 30 bp, Artificial Sequence
  Primer
ctaagcttctagataagatatccgatccac

SEQ ID NO: 54 - DNA, 31 bp, Artificial Sequence
  Primer
cgcgtcgacggtaccagatctctagcggatc

SEQ ID NO: 55 - DNA, 41 bp, Artificial Sequence
  Primer
gatctggtaccgtcgacgcgatgtttgtgtttctggtgctg

SEQ ID NO: 56 - DNA, 41 bp, Artificial Sequence
  Primer
tatcttatctagaagcttagtcaggtatagtgcagtttcac

SEQ ID NO: 57 - DNA, 40 bp, Artificial Sequence
  Primer
gatctggtaccgtcgacgcgatgggcctgcccaacaacac

SEQ ID NO: 58 - DNA, 41 bp, Artificial Sequence
  Primer
tatcttatctagaagcttagtcaggggaaggtcttgtaggc

SEQ ID NO: 59 - DNA, 30 bp, Artificial Sequence; identical to SEQ ID NO: 53
  Primer

SEQ ID NO: 60 - DNA, 31 bp, Artificial Sequence; identical to SEQ ID NO: 54
  Primer

SEQ ID NO: 61 - DNA, 38 bp, Artificial Sequence
  Primer
gatctggtaccgtcgacgcgatgcaccagaagagaaca

SEQ ID NO: 62 - DNA, 44 bp, Artificial Sequence
  Primer
tatcttatctagaagcttagttattgttgactagcgcaccatgg